European Patent Application EP 4 667 486 A1, published December 24, 2025. Title: A composition for treating autoimmune diseases comprising CD38 or fragments thereof. Applicant: Dnt Co., Ltd. The sequence listing filed with the application follows.

SEQUENCE LISTING (36 sequences)

SEQ ID NO: 1 - protein, 13 aa, synthetic construct
  REGION 1..13: note = 13 mer (Mouse, Rat or Horse)
FLQCVKNPEHPSC

SEQ ID NO: 2 - protein, 13 aa, synthetic construct
  REGION 1..13: note = 13 mer (Human or Chimpaanze)
FLQCVKNPEDSSC

SEQ ID NO: 3 - protein, 13 aa, synthetic construct
  REGION 1..13: note = 13 mer (Dog)
LLQCVKNPEHSSC

SEQ ID NO: 4 - protein, 14 aa, synthetic construct
  REGION 1..14: note = 14 mer (Mouse, Rat or Horse)
RFLQCVKNPEHPSC

SEQ ID NO: 5 - protein, 14 aa, synthetic construct
  REGION 1..14: note = 14 mer (Human or Chimpaanze)
KFLQCVKNPEDSSC

SEQ ID NO: 6 - protein, 14 aa, synthetic construct
  REGION 1..14: note = 14 mer (Dog)
RLLQCVKNPEHSSC

SEQ ID NO: 7 - protein, 15 aa, synthetic construct
  REGION 1..15: note = 15 mer (Mouse or Rat)
RFLQCVKNPEHPSCR

SEQ ID NO: 8 - protein, 15 aa, synthetic construct
  REGION 1..15: note = 15 mer (Human or Chimpaanze)
KFLQCVKNPEDSSCT

SEQ ID NO: 9 - protein, 15 aa, synthetic construct
  REGION 1..15: note = 15 mer (Dog)
RLLQCVKNPEHSSCK

SEQ ID NO: 10 - protein, 15 aa, synthetic construct
  REGION 1..15: note = 15 mer (Horse)
RFLQCVKNPEHPSCT

SEQ ID NO: 11 - protein, 16 aa, synthetic construct
  REGION 1..16: note = 16 mer (Mouse)
RFLQCVKNPEHPSCRL

SEQ ID NO: 12 - protein, 16 aa, synthetic construct
  REGION 1..16: note = 16 mer (Rat)
RFLQCVKNPEHPSCRL

SEQ ID NO: 13 - protein, 16 aa, synthetic construct
  REGION 1..16: note = 16 mer (Human or Chimpaanze)
KFLQCVKNPEDSSCTS

SEQ ID NO: 14 - protein, 16 aa, synthetic construct
  REGION 1..16: note = 16 mer (Dog)
RLLQCVKNPEHSSCKY

SEQ ID NO: 15 - protein, 16 aa, synthetic construct
  REGION 1..16: note = 16 mer (Horse)
RFLQCVKNPEHPSCTS

SEQ ID NO: 16 - protein, 18 aa, synthetic construct
  REGION 1..18: note = 18 mer (Mouse)
RFLQCVKNPEHPSCRLNT

SEQ ID NO: 17 - protein, 18 aa, synthetic construct
  REGION 1..18: note = 18 mer (Rat)
RFLQCVKNPEHPSCRLNV

SEQ ID NO: 18 - protein, 18 aa, synthetic construct
  REGION 1..18: note = 18 mer (Human or Chimpaanze)
KFLQCVKNPEDSSCTSEI

SEQ ID NO: 19 - protein, 18 aa, synthetic construct
  REGION 1..18: note = 18 mer (Dog)
RLLQCVKNPEHSSCKYNL

SEQ ID NO: 20 - protein, 18 aa, synthetic construct
  REGION 1..18: note = 18 mer (Horse)
RFLQCVKNPEHPSCTSGI

SEQ ID NO: 21 - protein, 19 aa, synthetic construct
  REGION 1..19: note = 19 mer (Mouse)
ARFLQCVKNPEHPSCRLNT

SEQ ID NO: 22 - protein, 19 aa, synthetic construct
  REGION 1..19: note = 19 mer (Rat)
VRFLQCVKNPEHPSCRLNV

SEQ ID NO: 23 - protein, 19 aa, synthetic construct
  REGION 1..19: note = 19 mer (Human or Chimpaanze)
DKFLQCVKNPEDSSCTSEI

SEQ ID NO: 24 - protein, 19 aa, synthetic construct
  REGION 1..19: note = 19 mer (Dog)
VRLLQCVKNPEHSSCKYNL

SEQ ID NO: 25 - protein, 19 aa, synthetic construct
  REGION 1..19: note = 19 mer (Horse)
VRFLQCVKNPEHPSCTSGI

SEQ ID NO: 26 - protein, 39 aa, synthetic construct
  REGION 1..39: note = 39 mer (Mouse)
LKMIVQKRNMIFACVDNYRPARFLQCVKNPEHPSCRLNT

SEQ ID NO: 27 - protein, 39 aa, synthetic construct
  REGION 1..39: note = 39 mer (Rat)
LKSIVNKRNMIFACQDNYRPVRFLQCVKNPEHPSCRLNV

SEQ ID NO: 28 - protein, 39 aa, synthetic construct
  REGION 1..39: note = 39 mer (Human or Chimpaanze)
LESIISKRNIQFSCKNIYRPDKFLQCVKNPEDSSCTSEI

SEQ ID NO: 29 - protein, 39 aa, synthetic construct
  REGION 1..39: note = 39 mer (Dog)
LKQILKTRNIIFICQNNYRPVRLLQCVKNPEHSSCKYNL

SEQ ID NO: 30 - protein, 39 aa, synthetic construct
  REGION 1..39: note = 39 mer (Horse)
LKSIISERNITFTCQNNYRPVRFLQCVKNPEHPSCTSGI

SEQ ID NO: 31 - protein, 308 aa, synthetic construct
  REGION 1..308: note = full length sCD38 (Dog)
MANHRFSSVSEEEKPCCGISRKAQICLCVLFILLIVVGIAVPVGILMWRQPPKHKEWKGPGTTAHFYEILLGRCYTYTQVVRPEQRHTDCQKIGKAFTSAFLSKDPCGSTEQDYRPLMELTTQIVPCDKTVFWSKSSELAHDYTRVQRDMYTLEDTLLGYMADGLKWCGDTSSSEMNYQSCPHWREDCSNNSVSVFWNTVSKRFAEDACGVVHVVLNGSISNTFDEKSTFGRVEVFNLHPEKVHTLKAWVMHNIESVPSDSCSSSSVNNLKQILKTRNIIFICQNNYRPVRLLQCVKNPEHSSCKYNL

SEQ ID NO: 32 - protein, 309 aa, synthetic construct
  REGION 1..309: note = full length sCD38 (Horse)
MANHRFSPVSEGEQPCCDISRKAQICLCVVLSLLVLVIIAVVTAILMWPRSPPNHKEWQGSGTTAHFGDIVLGRCYTYTQIVRPELRDKDCQKIQEVFLKSFLSKDPCDATEQDYQPLIELANQTVPCNKTVFWSKTKELAHQYTRVQQALFTLENTLLGYIADDLSWCGDSGSSEINYQSCPTRRDNCSSNPVSVFWNTVSKRFAEDACGVVHVVLNGSLNEAFDRRSTFGRVEIHNLHPKKVHTLQAWVMHDIGGVRSDSCSSSSIRDLKSIISERNITFTCQNNYRPVRFLQCVKNPEHPSCTSGI

SEQ ID NO: 33 - protein, 304 aa, synthetic construct
  REGION 1..304: note = full length sCD38 (Mouse)
MANYEFSQVSGDRPGCRLSRKAQIGLGVGLLVLIALVVGIVVILLRPRSLLVWTGEPTTKHFSDIFLGRCLIYTQILRPEMRDQNCQEILSTFKGAFVSKNPCNITREDYAPLVKLVTQTIPCNKTLFWSKSKHLAHQYTWIQGKMFTLEDTLLGYIADDLRWCGDPSTSDMNYVSCPHWSENCPNNPITVFWKVISQKFAEDACGVVQVMLNGSLREPFYKNSTFGSVEVFSLDPNKVHKLQAWVMHDIEGASSNACSSSSLNELKMIVQKRNMIFACVDNYRPARFLQCVKNPEHPSCRLNT

SEQ ID NO: 34 - protein, 303 aa, synthetic construct
  REGION 1..303: note = full length sCD38 (Rat)
MANYEFSQVSEDRPGCRLTRKAQIGLGVGLLLLVALVVVVVIVLWPRSPLVWKGKPTTKHFADIILGRCLIYTQILRPEMRDQDCKKILSTFKRGFISKNPCNITNEDYAPLVKLVTQTIPCNKTLFWSKSKHLAHQYTWIQGKMFTLEDTLLGYIADDLRWCGDPSTSDMNYDSCPHWSENCPNNPVAVFWNVISQKFAEDACGVVQVMLNGSLSEPFYRNSTFGSVEVFNLDPNKVHKLQAWVMHDIKGTSSNACSSPSINELKSIVNKRNMIFACQDNYRPVRFLQCVKNPEHPSCRLNV

SEQ ID NO: 35 - protein, 300 aa, synthetic construct
  REGION 1..300: note = full length sCD38 (Human)
MANCEFSPVSGDKPCCRLSRRAQLCLGVSILVLILVVVLAVVVPRWRQQWSGPGTTKRFPETVLARCVKYTEIHPEMRHVDCQSVWDAFKGAFISKHPCNITEEDYQPLMKLGTQTVPCNKILLWSRIKDLAHQFTQVQRDMFTLEDTLLGYLADDLTWCGEFNTSKINYQSCPDWRKDCSNNPVSVFWKTVSRRFAEAACDVVHVMLNGSRSKIFDKNSTFGSVEVHNLQPEKVQTLEAWVIHGGREDSRDLCQDPTIKELESIISKRNIQFSCKNIYRPDKFLQCVKNPEDSSCTSEI

SEQ ID NO: 36 - protein, 300 aa, synthetic construct
  REGION 1..300: note = full length sCD38 (Chimpaanze)
MANCEFSPVSGDKPCCRLSRRAQLCLGVSILVLILVVVLAVVVPRWRQQWSGPGTTKRFPETVLARCVKYTEIHPEMRHVDCQSVWDAFKGAFISKHPCNITEEDYQPLMKLGTQTVPCNKILLWSRIKDLAHQFTQVQQDMFTLEDTLLGYLADDLTWCGEFSTSEINYQSCPDWRKDCSNNPVSVFWKTVSRRFAEAACDVVHVMLNGSRSKIFDKNSTFGSVEVHNLQPEKVQTLEAWVIHGGREDSRDLCQDPTIKELESIISKRNIQFSCKNIYRPDKFLQCVKNPEDSSCTSEI